European Patent Application EP 4 477 670 A1, published December 18, 2024. Title: BISPECIFIC ANTIGEN-BINDING MOLECULE AND USE THEREOF. Applicant: Shanghai Qilu Pharmaceutical Research and Development Centre Ltd. Application CN PCT/CN2023/075148, filed February 9, 2023. The sequence listing filed with the application follows.

SEQUENCE LISTING (34 sequences)

SEQ ID NO: 1 - protein, 613 aa, synthetic construct
EVQLVESGGGLVQPGGSLRLSCAASTYTISSGYMGWFRQAPGKEREGVAAIYIGGSTTLYADSVKGRFTISRDNSKNTLYLQMNSLRAEDTAVYYCAAQLRPNAAYHPLDGRKYNYWGQGTLVTVSSGGGGSEVKLVESGGGLVQPGGSLKLSCAASGFTFNTYAMNWVRQAPGKGLEWVARIRSKYNNYATYYADSVKDRFTISRDDAKNTLYLQMNNLRTEDTAVYYCVRHGNFGNSYVSWFAYWGQGTLVTVSSGGGGSGGGGSGGGGSQAVVTQEPSLTVSPGGTVTLTCRSSTGAVTTSNYANWVQQKPGQAPRGLIGGTNKRAPGTPARFSGSLLGGKAALTLSGAQPEDEAEYYCALWYSNLWVFGGGTKLTVLEPKSSDKTHTCPPCPAPEAAGGPSVFLFPPKPKDTLMISRTPEVTCVVVDVSHEDPEVKFNWYVDGVEVHNAKTKPREEQYNSTYRVVSVLTVLHQDWLNGKEYKCKVSNKALPAPIEKTISKAKGQPREPQVYTLPPSRDELTKNQVSLTCLVKGFYPSDIAVEWESNGQPENNYKTTPPVLDSDGSFFLYSKLTVDKSRWQQGNVFSCSVMHEALHNHYTQKSLSLSPGK

SEQ ID NO: 2 - protein, 721 aa, synthetic construct
QVQLVQSGAEVKKPGASVKVSCKASGYTFISYWITWVRQAPGQGLEWMGDIYPGSGSTTNYNEKFKSRVTMTRDTSTSTVYMELSSLRSEDTAVYYCARETTVGGAYAMDYWGQGTLVTVSSASTKGPSVFPLAPSSKSTSGGTAALGCLVKDYFPEPVTVSWNSGALTSGVHTFPAVLQSSGLYSLSSVVTVPSSSLGTQTYICNVNHKPSNTKVDKKVEPKSCGGGGSGGGGSGGGGSEVKLVESGGGLVQPGGSLKLSCAASGFTFNTYAMNWVRQAPGKGLEWVARIRSKYNNYATYYADSVKDRFTISRDDAKNTLYLQMNNLRTEDTAVYYCVRHGNFGNSYVSWFAYWGQGTLVTVSSGGGGSGGGGSGGGGSQAVVTQEPSLTVSPGGTVTLTCRSSTGAVTTSNYANWVQQKPGQAPRGLIGGTNKRAPGTPARFSGSLLGGKAALTLSGAQPEDEAEYYCALWYSNLWVFGGGTKLTVLEPKSSDKTHTCPPCPAPEAAGGPSVFLFPPKPKDTLMISRTPEVTCVVVDVSHEDPEVKFNWYVDGVEVHNAKTKPREEQYNSTYRVVSVLTVLHQDWLNGKEYKCKVSNKALPAPIEKTISKAKGQPREPQVYTLPPCRDELTKNQVSLWCLVKGFYPSDIAVEWESNGQPENNYKTTPPVLDSDGSFFLYSKLTVDKSRWQQGNVFSCSVMHEALHNHYTQKSLSLSPGK

SEQ ID NO: 3 - protein, 227 aa, synthetic construct
DKTHTCPPCPAPEAAGGPSVFLFPPKPKDTLMISRTPEVTCVVVDVSHEDPEVKFNWYVDGVEVHNAKTKPREEQYNSTYRVVSVLTVLHQDWLNGKEYKCKVSNKALPAPIEKTISKAKGQPREPQVCTLPPSRDELTKNQVSLSCAVKGFYPSDIAVEWESNGQPENNYKTTPPVLDSDGSFFLVSKLTVDKSRWQQGNVFSCSVMHEALHNRYTQKSLSLSPGK

SEQ ID NO: 4 - protein, 214 aa, synthetic construct
EIVLTQSPATLSLSPGERATLSCRASQSINNNLHWYQQKPGQAPRLLIKYVSQSISGIPARFSGSGSGTDFTLTISSLEPEDFAVYYCQQTNAWPLTFGGGTKLEIKRTVAAPSVFIFPPSDEQLKSGTASVVCLLNNFYPREAKVQWKVDNALQSGNSQESVTEQDSKDSTYSLSSTLTLSKADYEKHKVYACEVTHQGLSSPVTKSFNRGEC

SEQ ID NO: 5 - protein, 358 aa, synthetic construct
EVQLVESGGGLVQPGGSLRLSCAASTYTISSGYMGWFRQAPGKEREGVAAIYIGGSTTLYADSVKGRFTISRDNSKNTLYLQMNSLRAEDTAVYYCAAQLRPNAAYHPLDGRKYNYWGQGTLVTVSSGGGGSDKTHTCPPCPAPELLGGPSVFLFPPKPKDTLMISRTPEVTCVVVDVSHEDPEVKFNWYVDGVEVHNAKTKPREEQYNSTYRVVSVLTVLHQDWLNGKEYKCKVSNKALPAPIEKTISKAKGQPREPQVYTLPPSRDELTKNQVSLTCLVKGFYPSDIAVEWESNGQPENNYKTTPPVLDSDGSFFLYSKLTVDKSRWQQGNVFSCSVMHEALHNHYTQKSLSLSPG

SEQ ID NO: 6 - protein, 5 aa, synthetic construct
SGYMG

SEQ ID NO: 7 - protein, 18 aa, synthetic construct
AAIYIGGSTTLYADSVKG

SEQ ID NO: 8 - protein, 18 aa, synthetic construct
QLRPNAAYHPLDGRKYNY

SEQ ID NO: 9 - protein, 452 aa, synthetic construct
QVQLVQSGAEVKKPGASVKVSCKASGYTFISYWITWVRQAPGQGLEWMGDIYPGSGSTTNYNEKFKSRVTMTRDTSTSTVYMELSSLRSEDTAVYYCARETTVGGAYAMDYWGQGTLVTVSSASTKGPSVFPLAPSSKSTSGGTAALGCLVKDYFPEPVTVSWNSGALTSGVHTFPAVLQSSGLYSLSSVVTVPSSSLGTQTYICNVNHKPSNTKVDKKVEPKSCDKTHTCPPCPAPELLGGPSVFLFPPKPKDTLMISRTPEVTCVVVDVSHEDPEVKFNWYVDGVEVHNAKTKPREEQYNSTYRVVSVLTVLHQDWLNGKEYKCKVSNKALPAPIEKTISKAKGQPREPQVYTLPPSRDELTKNQVSLTCLVKGFYPSDIAVEWESNGQPENNYKTTPPVLDSDGSFFLYSKLTVDKSRWQQGNVFSCSVMHEALHNHYTQKSLSLSPGK

SEQ ID NO: 10 - protein, 214 aa, synthetic construct; identical to SEQ ID NO: 4

SEQ ID NO: 11 - protein, 122 aa, synthetic construct
QVQLVQSGAEVKKPGASVKVSCKASGYTFISYWITWVRQAPGQGLEWMGDIYPGSGSTTNYNEKFKSRVTMTRDTSTSTVYMELSSLRSEDTAVYYCARETTVGGAYAMDYWGQGTLVTVSS

SEQ ID NO: 12 - protein, 107 aa, synthetic construct
EIVLTQSPATLSLSPGERATLSCRASQSINNNLHWYQQKPGQAPRLLIKYVSQSISGIPARFSGSGSGTDFTLTISSLEPEDFAVYYCQQTNAWPLTFGGGTKLEIK

SEQ ID NO: 13 - protein, 5 aa, synthetic construct
SYWIT

SEQ ID NO: 14 - protein, 18 aa, synthetic construct
DIYPGSGSTTNYNEKFKS

SEQ ID NO: 15 - protein, 12 aa, synthetic construct
ETTVGGAYAMDY

SEQ ID NO: 16 - protein, 11 aa, synthetic construct
RASQSINNNLH

SEQ ID NO: 17 - protein, 7 aa, synthetic construct
YVSQSIS

SEQ ID NO: 18 - protein, 9 aa, synthetic construct
QQTNAWPLT

SEQ ID NO: 19 - protein, 455 aa, synthetic construct
EVKLVESGGGLVQPGGSLKLSCAASGFTFNTYAMNWVRQAPGKGLEWVARIRSKYNNYATYYADSVKDRFTISRDDAKNTLYLQMNNLRTEDTAVYYCVRHGNFGNSYVSWFAYWGQGTLVTVSSASTKGPSVFPLAPSSKSTSGGTAALGCLVKDYFPEPVTVSWNSGALTSGVHTFPAVLQSSGLYSLSSVVTVPSSSLGTQTYICNVNHKPSNTKVDKKVEPKSCDKTHTCPPCPAPEAAGGPSVFLFPPKPKDTLMISRTPEVTCVVVDVSHEDPEVKFNWYVDGVEVHNAKTKPREEQYNSTYRVVSVLTVLHQDWLNGKEYKCKVSNKALPAPIEKTISKAKGQPREPQVYTLPPSRDELTKNQVSLTCLVKGFYPSDIAVEWESNGQPENNYKTTPPVLDSDGSFFLYSKLTVDKSRWQQGNVFSCSVMHEALHNHYTQKSLSLSPGK

SEQ ID NO: 20 - protein, 214 aa, synthetic construct
QAVVTQEPSLTVSPGGTVTLTCRSSTGAVTTSNYANWVQQKPGQAPRGLIGGTNKRAPGTPARFSGSLLGGKAALTLSGAQPEDEAEYYCALWYSNLWVFGGGTKLTVLGQPKANPTVTLFPPSSEELQANKATLVCLISDFYPGAVTVAWKADSSPVKAGVETTTPSKQSNNKYAASSYLSLTPEQWKSHRSYSCQVTHEGSTVEKTVAPTEC

SEQ ID NO: 21 - protein, 125 aa, synthetic construct
EVKLVESGGGLVQPGGSLKLSCAASGFTFNTYAMNWVRQAPGKGLEWVARIRSKYNNYATYYADSVKDRFTISRDDAKNTLYLQMNNLRTEDTAVYYCVRHGNFGNSYVSWFAYWGQGTLVTVSS

SEQ ID NO: 22 - protein, 109 aa, synthetic construct
QAVVTQEPSLTVSPGGTVTLTCRSSTGAVTTSNYANWVQQKPGQAPRGLIGGTNKRAPGTPARFSGSLLGGKAALTLSGAQPEDEAEYYCALWYSNLWVFGGGTKLTVL

SEQ ID NO: 23 - protein, 249 aa, synthetic construct
EVKLVESGGGLVQPGGSLKLSCAASGFTFNTYAMNWVRQAPGKGLEWVARIRSKYNNYATYYADSVKDRFTISRDDAKNTLYLQMNNLRTEDTAVYYCVRHGNFGNSYVSWFAYWGQGTLVTVSSGGGGSGGGGSGGGGSQAVVTQEPSLTVSPGGTVTLTCRSSTGAVTTSNYANWVQQKPGQAPRGLIGGTNKRAPGTPARFSGSLLGGKAALTLSGAQPEDEAEYYCALWYSNLWVFGGGTKLTVL

SEQ ID NO: 24 - protein, 5 aa, synthetic construct
TYAMN

SEQ ID NO: 25 - protein, 19 aa, synthetic construct
RIRSKYNNYATYYADSVKD

SEQ ID NO: 26 - protein, 14 aa, synthetic construct
HGNFGNSYVSWFAY

SEQ ID NO: 27 - protein, 14 aa, synthetic construct
RSSTGAVTTSNYAN

SEQ ID NO: 28 - protein, 7 aa, synthetic construct
GTNKRAP

SEQ ID NO: 29 - protein, 9 aa, synthetic construct
ALWYSNLWV

SEQ ID NO: 30 - protein, 227 aa, synthetic construct
DKTHTCPPCPAPEAAGGPSVFLFPPKPKDTLMISRTPEVTCVVVDVSHEDPEVKFNWYVDGVEVHNAKTKPREEQYNSTYRVVSVLTVLHQDWLNGKEYKCKVSNKALPAPIEKTISKAKGQPREPQVYTLPPSRDELTKNQVSLTCLVKGFYPSDIAVEWESNGQPENNYKTTPPVLDSDGSFFLYSKLTVDKSRWQQGNVFSCSVMHEALHNHYTQKSLSLSPGK

SEQ ID NO: 31 - protein, 227 aa, synthetic construct
DKTHTCPPCPAPEAAGGPSVFLFPPKPKDTLMISRTPEVTCVVVDVSHEDPEVKFNWYVDGVEVHNAKTKPREEQYNSTYRVVSVLTVLHQDWLNGKEYKCKVSNKALPAPIEKTISKAKGQPREPQVYTLPPCRDELTKNQVSLWCLVKGFYPSDIAVEWESNGQPENNYKTTPPVLDSDGSFFLYSKLTVDKSRWQQGNVFSCSVMHEALHNHYTQKSLSLSPGK

SEQ ID NO: 32 - protein, 127 aa, synthetic construct
EVQLVESGGGLVQPGGSLRLSCAASTYTISSGYMGWFRQAPGKEREGVAAIYIGGSTTLYADSVKGRFTISRDNSKNTLYLQMNSLRAEDTAVYYCAAQLRPNAAYHPLDGRKYNYWGQGTLVTVSS

SEQ ID NO: 33 - protein, 225 aa, synthetic construct
QVQLVQSGAEVKKPGASVKVSCKASGYTFISYWITWVRQAPGQGLEWMGDIYPGSGSTTNYNEKFKSRVTMTRDTSTSTVYMELSSLRSEDTAVYYCARETTVGGAYAMDYWGQGTLVTVSSASTKGPSVFPLAPSSKSTSGGTAALGCLVKDYFPEPVTVSWNSGALTSGVHTFPAVLQSSGLYSLSSVVTVPSSSLGTQTYICNVNHKPSNTKVDKKVEPKSC

SEQ ID NO: 34 - protein, 5 aa, synthetic construct
EPKSS